European Patent Application EP 4 140 498 A1, published March 1, 2023. Title: 一种治疗脊髓性肌萎缩症的方法和药物. Applicant: 泰伦基国际有限公司. The sequence listing filed with the application follows.

SEQUENCE LISTING (16 sequences)

SEQ ID NO: 1 - DNA, 2376 bp, 人工序列
  人工序列的描述：合成的多核苷酸
  不含有信号肽的天然纤溶酶原(Glu-PLG，Glu-纤维蛋白溶酶原)核酸序列
gagcctctggatgactatgtgaatacccagggggcttcactgttcagtgtcactaagaagcagctgggagcaggaagtatagaagaatgtgcagcaaaatgtgaggaggacgaagaattcacctgcagggcattccaatatcacagtaaagagcaacaatgtgtgataatggctgaaaacaggaagtcctccataatcattaggatgagagatgtagttttatttgaaaagaaagtgtatctctcagagtgcaagactgggaatggaaagaactacagagggacgatgtccaaaacaaaaaatggcatcacctgtcaaaaatggagttccacttctccccacagacctagattctcacctgctacacacccctcagagggactggaggagaactactgcaggaatccagacaacgatccgcaggggccctggtgctatactactgatccagaaaagagatatgactactgcgacattcttgagtgtgaagaggaatgtatgcattgcagtggagaaaactatgacggcaaaatttccaagaccatgtctggactggaatgccaggcctgggactctcagagcccacacgctcatggatacattccttccaaatttccaaacaagaacctgaagaagaattactgtcgtaaccccgatagggagctgcggccttggtgtttcaccaccgaccccaacaagcgctgggaactttgtgacatcccccgctgcacaacacctccaccatcttctggtcccacctaccagtgtctgaagggaacaggtgaaaactatcgcgggaatgtggctgttaccgtgtccgggcacacctgtcagcactggagtgcacagacccctcacacacataacaggacaccagaaaacttcccctgcaaaaatttggatgaaaactactgccgcaatcctgacggaaaaagggccccatggtgccatacaaccaacagccaagtgcggtgggagtactgtaagataccgtcctgtgactcctccccagtatccacggaacaattggctcccacagcaccacctgagctaacccctgtggtccaggactgctaccatggtgatggacagagctaccgaggcacatcctccaccaccaccacaggaaagaagtgtcagtcttggtcatctatgacaccacaccggcaccagaagaccccagaaaactacccaaatgctggcctgacaatgaactactgcaggaatccagatgccgataaaggcccctggtgttttaccacagaccccagcgtcaggtgggagtactgcaacctgaaaaaatgctcaggaacagaagcgagtgttgtagcacctccgcctgttgtcctgcttccagatgtagagactccttccgaagaagactgtatgtttgggaatgggaaaggataccgaggcaagagggcgaccactgttactgggacgccatgccaggactgggctgcccaggagccccatagacacagcattttcactccagagacaaatccacgggcgggtctggaaaaaaattactgccgtaaccctgatggtgatgtaggtggtccctggtgctacacgacaaatccaagaaaactttacgactactgtgatgtccctcagtgtgcggccccttcatttgattgtgggaagcctcaagtggagccgaagaaatgtcctggaagggttgtaggggggtgtgtggcccacccacattcctggccctggcaagtcagtcttagaacaaggtttggaatgcacttctgtggaggcaccttgatatccccagagtgggtgttgactgctgcccactgcttggagaagtccccaaggccttcatcctacaaggtcatcctgggtgcacaccaagaagtgaatctcgaaccgcatgttcaggaaatagaagtgtctaggctgttcttggagcccacacgaaaagatattgccttgctaaagctaagcagtcctgccgtcatcactgacaaagtaatcccagcttgtctgccatccccaaattatgtggtcgctgaccggaccgaatgtttcatcactggctggggagaaacccaaggtacttttggagctggccttctcaaggaagcccagctccctgtgattgagaataaagtgtgcaatcgctatgagtttctgaatggaagagtccaatccaccgaactctgtgctgggcatttggccggaggcactgacagttgccagggtgacagtggaggtcctctggtttgcttcgagaaggacaaatacattttacaaggagtcacttcttggggtcttggctgtgcacgccccaataagcctggtgtctatgttcgtgtttcaaggtttgttacttggattgagggagtgatgagaaataattaa

SEQ ID NO: 2 - protein, 791 aa, 人工序列
  人工序列的描述：合成的多肽
  不含有信号肽的天然纤溶酶原(Glu-PLG，Glu-纤维蛋白溶酶原)核酸序列
EPLDDYVNTQGASLFSVTKKQLGAGSIEECAAKCEEDEEFTCRAFQYHSKEQQCVIMAENRKSSIIIRMRDVVLFEKKVYLSECKTGNGKNYRGTMSKTKNGITCQKWSSTSPHRPRFSPATHPSEGLEENYCRNPDNDPQGPWCYTTDPEKRYDYCDILECEEECMHCSGENYDGKISKTMSGLECQAWDSQSPHAHGYIPSKFPNKNLKKNYCRNPDRELRPWCFTTDPNKRWELCDIPRCTTPPPSSGPTYQCLKGTGENYRGNVAVTVSGHTCQHWSAQTPHTHNRTPENFPCKNLDENYCRNPDGKRAPWCHTTNSQVRWEYCKIPSCDSSPVSTEQLAPTAPPELTPVVQDCYHGDGQSYRGTSSTTTTGKKCQSWSSMTPHRHQKTPENYPNAGLTMNYCRNPDADKGPWCFTTDPSVRWEYCNLKKCSGTEASVVAPPPVVLLPDVETPSEEDCMFGNGKGYRGKRATTVTGTPCQDWAAQEPHRHSIFTPETNPRAGLEKNYCRNPDGDVGGPWCYTTNPRKLYDYCDVPQCAAPSFDCGKPQVEPKKCPGRVVGGCVAHPHSWPWQVSLRTRFGMHFCGGTLISPEWVLTAAHCLEKSPRPSSYKVILGAHQEVNLEPHVQEIEVSRLFLEPTRKDIALLKLSSPAVITDKVIPACLPSPNYVVADRTECFITGWGETQGTFGAGLLKEAQLPVIENKVCNRYEFLNGRVQSTELCAGHLAGGTDSCQGDSGGPLVCFEKDKYILQGVTSWGLGCARPNKPGVYVRVSRFVTWIEGVMRNN

SEQ ID NO: 3 - DNA, 2433 bp, 人工序列
  人工序列的描述：合成的多核苷酸
  含有信号肽的天然纤溶酶原(来源于swiss prot)的核酸序列
atggaacataaggaagtggttcttctacttcttttatttctgaaatcaggtcaaggagagcctctggatgactatgtgaatacccagggggcttcactgttcagtgtcactaagaagcagctgggagcaggaagtatagaagaatgtgcagcaaaatgtgaggaggacgaagaattcacctgcagggcattccaatatcacagtaaagagcaacaatgtgtgataatggctgaaaacaggaagtcctccataatcattaggatgagagatgtagttttatttgaaaagaaagtgtatctctcagagtgcaagactgggaatggaaagaactacagagggacgatgtccaaaacaaaaaatggcatcacctgtcaaaaatggagttccacttctccccacagacctagattctcacctgctacacacccctcagagggactggaggagaactactgcaggaatccagacaacgatccgcaggggccctggtgctatactactgatccagaaaagagatatgactactgcgacattcttgagtgtgaagaggaatgtatgcattgcagtggagaaaactatgacggcaaaatttccaagaccatgtctggactggaatgccaggcctgggactctcagagcccacacgctcatggatacattccttccaaatttccaaacaagaacctgaagaagaattactgtcgtaaccccgatagggagctgcggccttggtgtttcaccaccgaccccaacaagcgctgggaactttgtgacatcccccgctgcacaacacctccaccatcttctggtcccacctaccagtgtctgaagggaacaggtgaaaactatcgcgggaatgtggctgttaccgtgtccgggcacacctgtcagcactggagtgcacagacccctcacacacataacaggacaccagaaaacttcccctgcaaaaatttggatgaaaactactgccgcaatcctgacggaaaaagggccccatggtgccatacaaccaacagccaagtgcggtgggagtactgtaagataccgtcctgtgactcctccccagtatccacggaacaattggctcccacagcaccacctgagctaacccctgtggtccaggactgctaccatggtgatggacagagctaccgaggcacatcctccaccaccaccacaggaaagaagtgtcagtcttggtcatctatgacaccacaccggcaccagaagaccccagaaaactacccaaatgctggcctgacaatgaactactgcaggaatccagatgccgataaaggcccctggtgttttaccacagaccccagcgtcaggtgggagtactgcaacctgaaaaaatgctcaggaacagaagcgagtgttgtagcacctccgcctgttgtcctgcttccagatgtagagactccttccgaagaagactgtatgtttgggaatgggaaaggataccgaggcaagagggcgaccactgttactgggacgccatgccaggactgggctgcccaggagccccatagacacagcattttcactccagagacaaatccacgggcgggtctggaaaaaaattactgccgtaaccctgatggtgatgtaggtggtccctggtgctacacgacaaatccaagaaaactttacgactactgtgatgtccctcagtgtgcggccccttcatttgattgtgggaagcctcaagtggagccgaagaaatgtcctggaagggttgtaggggggtgtgtggcccacccacattcctggccctggcaagtcagtcttagaacaaggtttggaatgcacttctgtggaggcaccttgatatccccagagtgggtgttgactgctgcccactgcttggagaagtccccaaggccttcatcctacaaggtcatcctgggtgcacaccaagaagtgaatctcgaaccgcatgttcaggaaatagaagtgtctaggctgttcttggagcccacacgaaaagatattgccttgctaaagctaagcagtcctgccgtcatcactgacaaagtaatcccagcttgtctgccatccccaaattatgtggtcgctgaccggaccgaatgtttcatcactggctggggagaaacccaaggtacttttggagctggccttctcaaggaagcccagctccctgtgattgagaataaagtgtgcaatcgctatgagtttctgaatggaagagtccaatccaccgaactctgtgctgggcatttggccggaggcactgacagttgccagggtgacagtggaggtcctctggtttgcttcgagaaggacaaatacattttacaaggagtcacttcttggggtcttggctgtgcacgccccaataagcctggtgtctatgttcgtgtttcaaggtttgttacttggattgagggagtgatgagaaataattaa

SEQ ID NO: 4 - protein, 810 aa, 人工序列
  人工序列的描述：合成的多肽
  含有信号肽的天然纤溶酶原(来源于swiss prot)的氨基酸序列
MEHKEVVLLLLLFLKSGQGEPLDDYVNTQGASLFSVTKKQLGAGSIEECAAKCEEDEEFTCRAFQYHSKEQQCVIMAENRKSSIIIRMRDVVLFEKKVYLSECKTGNGKNYRGTMSKTKNGITCQKWSSTSPHRPRFSPATHPSEGLEENYCRNPDNDPQGPWCYTTDPEKRYDYCDILECEEECMHCSGENYDGKISKTMSGLECQAWDSQSPHAHGYIPSKFPNKNLKKNYCRNPDRELRPWCFTTDPNKRWELCDIPRCTTPPPSSGPTYQCLKGTGENYRGNVAVTVSGHTCQHWSAQTPHTHNRTPENFPCKNLDENYCRNPDGKRAPWCHTTNSQVRWEYCKIPSCDSSPVSTEQLAPTAPPELTPVVQDCYHGDGQSYRGTSSTTTTGKKCQSWSSMTPHRHQKTPENYPNAGLTMNYCRNPDADKGPWCFTTDPSVRWEYCNLKKCSGTEASVVAPPPVVLLPDVETPSEEDCMFGNGKGYRGKRATTVTGTPCQDWAAQEPHRHSIFTPETNPRAGLEKNYCRNPDGDVGGPWCYTTNPRKLYDYCDVPQCAAPSFDCGKPQVEPKKCPGRVVGGCVAHPHSWPWQVSLRTRFGMHFCGGTLISPEWVLTAAHCLEKSPRPSSYKVILGAHQEVNLEPHVQEIEVSRLFLEPTRKDIALLKLSSPAVITDKVIPACLPSPNYVVADRTECFITGWGETQGTFGAGLLKEAQLPVIENKVCNRYEFLNGRVQSTELCAGHLAGGTDSCQGDSGGPLVCFEKDKYILQGVTSWGLGCARPNKPGVYVRVSRFVTWIEGVMRNN

SEQ ID NO: 5 - DNA, 2145 bp, 人工序列
  人工序列的描述：合成的多核苷酸
  LYS77-PLG(Lys-纤溶酶原)核酸序列
aaagtgtatctctcagagtgcaagactgggaatggaaagaactacagagggacgatgtccaaaacaaaaaatggcatcacctgtcaaaaatggagttccacttctccccacagacctagattctcacctgctacacacccctcagagggactggaggagaactactgcaggaatccagacaacgatccgcaggggccctggtgctatactactgatccagaaaagagatatgactactgcgacattcttgagtgtgaagaggaatgtatgcattgcagtggagaaaactatgacggcaaaatttccaagaccatgtctggactggaatgccaggcctgggactctcagagcccacacgctcatggatacattccttccaaatttccaaacaagaacctgaagaagaattactgtcgtaaccccgatagggagctgcggccttggtgtttcaccaccgaccccaacaagcgctgggaactttgtgacatcccccgctgcacaacacctccaccatcttctggtcccacctaccagtgtctgaagggaacaggtgaaaactatcgcgggaatgtggctgttaccgtgtccgggcacacctgtcagcactggagtgcacagacccctcacacacataacaggacaccagaaaacttcccctgcaaaaatttggatgaaaactactgccgcaatcctgacggaaaaagggccccatggtgccatacaaccaacagccaagtgcggtgggagtactgtaagataccgtcctgtgactcctccccagtatccacggaacaattggctcccacagcaccacctgagctaacccctgtggtccaggactgctaccatggtgatggacagagctaccgaggcacatcctccaccaccaccacaggaaagaagtgtcagtcttggtcatctatgacaccacaccggcaccagaagaccccagaaaactacccaaatgctggcctgacaatgaactactgcaggaatccagatgccgataaaggcccctggtgttttaccacagaccccagcgtcaggtgggagtactgcaacctgaaaaaatgctcaggaacagaagcgagtgttgtagcacctccgcctgttgtcctgcttccagatgtagagactccttccgaagaagactgtatgtttgggaatgggaaaggataccgaggcaagagggcgaccactgttactgggacgccatgccaggactgggctgcccaggagccccatagacacagcattttcactccagagacaaatccacgggcgggtctggaaaaaaattactgccgtaaccctgatggtgatgtaggtggtccctggtgctacacgacaaatccaagaaaactttacgactactgtgatgtccctcagtgtgcggccccttcatttgattgtgggaagcctcaagtggagccgaagaaatgtcctggaagggttgtaggggggtgtgtggcccacccacattcctggccctggcaagtcagtcttagaacaaggtttggaatgcacttctgtggaggcaccttgatatccccagagtgggtgttgactgctgcccactgcttggagaagtccccaaggccttcatcctacaaggtcatcctgggtgcacaccaagaagtgaatctcgaaccgcatgttcaggaaatagaagtgtctaggctgttcttggagcccacacgaaaagatattgccttgctaaagctaagcagtcctgccgtcatcactgacaaagtaatcccagcttgtctgccatccccaaattatgtggtcgctgaccggaccgaatgtttcatcactggctggggagaaacccaaggtacttttggagctggccttctcaaggaagcccagctccctgtgattgagaataaagtgtgcaatcgctatgagtttctgaatggaagagtccaatccaccgaactctgtgctgggcatttggccggaggcactgacagttgccagggtgacagtggaggtcctctggtttgcttcgagaaggacaaatacattttacaaggagtcacttcttggggtcttggctgtgcacgccccaataagcctggtgtctatgttcgtgtttcaaggtttgttacttggattgagggagtgatgagaaataattaa

SEQ ID NO: 6 - protein, 714 aa, 人工序列
  人工序列的描述：合成的多肽
  LYS77-PLG(Lys-纤溶酶原)氨基酸序列
KVYLSECKTGNGKNYRGTMSKTKNGITCQKWSSTSPHRPRFSPATHPSEGLEENYCRNPDNDPQGPWCYTTDPEKRYDYCDILECEEECMHCSGENYDGKISKTMSGLECQAWDSQSPHAHGYIPSKFPNKNLKKNYCRNPDRELRPWCFTTDPNKRWELCDIPRCTTPPPSSGPTYQCLKGTGENYRGNVAVTVSGHTCQHWSAQTPHTHNRTPENFPCKNLDENYCRNPDGKRAPWCHTTNSQVRWEYCKIPSCDSSPVSTEQLAPTAPPELTPVVQDCYHGDGQSYRGTSSTTTTGKKCQSWSSMTPHRHQKTPENYPNAGLTMNYCRNPDADKGPWCFTTDPSVRWEYCNLKKCSGTEASVVAPPPVVLLPDVETPSEEDCMFGNGKGYRGKRATTVTGTPCQDWAAQEPHRHSIFTPETNPRAGLEKNYCRNPDGDVGGPWCYTTNPRKLYDYCDVPQCAAPSFDCGKPQVEPKKCPGRVVGGCVAHPHSWPWQVSLRTRFGMHFCGGTLISPEWVLTAAHCLEKSPRPSSYKVILGAHQEVNLEPHVQEIEVSRLFLEPTRKDIALLKLSSPAVITDKVIPACLPSPNYVVADRTECFITGWGETQGTFGAGLLKEAQLPVIENKVCNRYEFLNGRVQSTELCAGHLAGGTDSCQGDSGGPLVCFEKDKYILQGVTSWGLGCARPNKPGVYVRVSRFVTWIEGVMRNN

SEQ ID NO: 7 - DNA, 1245 bp, 人工序列
  人工序列的描述：合成的多核苷酸
  delta-plg(delta-纤溶酶原)核酸序列
gagcctctggatgactatgtgaatacccagggggcttcactgttcagtgtcactaagaagcagctgggagcaggaagtatagaagaatgtgcagcaaaatgtgaggaggacgaagaattcacctgcagggcattccaatatcacagtaaagagcaacaatgtgtgataatggctgaaaacaggaagtcctccataatcattaggatgagagatgtagttttatttgaaaagaaagtgtatctctcagagtgcaagactgggaatggaaagaactacagagggacgatgtccaaaacaaaaaatggcatcacctgtcaaaaatggagttccacttctccccacagacctagattctcacctgctacacacccctcagagggactggaggagaactactgcaggaatccagacaacgatccgcaggggccctggtgctatactactgatccagaaaagagatatgactactgcgacattcttgagtgtgaagaggcggccccttcatttgattgtgggaagcctcaagtggagccgaagaaatgtcctggaagggttgtaggggggtgtgtggcccacccacattcctggccctggcaagtcagtcttagaacaaggtttggaatgcacttctgtggaggcaccttgatatccccagagtgggtgttgactgctgcccactgcttggagaagtccccaaggccttcatcctacaaggtcatcctgggtgcacaccaagaagtgaatctcgaaccgcatgttcaggaaatagaagtgtctaggctgttcttggagcccacacgaaaagatattgccttgctaaagctaagcagtcctgccgtcatcactgacaaagtaatcccagcttgtctgccatccccaaattatgtggtcgctgaccggaccgaatgtttcatcactggctggggagaaacccaaggtacttttggagctggccttctcaaggaagcccagctccctgtgattgagaataaagtgtgcaatcgctatgagtttctgaatggaagagtccaatccaccgaactctgtgctgggcatttggccggaggcactgacagttgccagggtgacagtggaggtcctctggtttgcttcgagaaggacaaatacattttacaaggagtcacttcttggggtcttggctgtgcacgccccaataagcctggtgtctatgttcgtgtttcaaggtttgttacttggattgagggagtgatgagaaataattaa

SEQ ID NO: 8 - protein, 414 aa, 人工序列
  人工序列的描述：合成的多肽
  delta-plg(delta-纤溶酶原)氨基酸序列
EPLDDYVNTQGASLFSVTKKQLGAGSIEECAAKCEEDEEFTCRAFQYHSKEQQCVIMAENRKSSIIIRMRDVVLFEKKVYLSECKTGNGKNYRGTMSKTKNGITCQKWSSTSPHRPRFSPATHPSEGLEENYCRNPDNDPQGPWCYTTDPEKRYDYCDILECEEAAPSFDCGKPQVEPKKCPGRVVGGCVAHPHSWPWQVSLRTRFGMHFCGGTLISPEWVLTAAHCLEKSPRPSSYKVILGAHQEVNLEPHVQEIEVSRLFLEPTRKDIALLKLSSPAVITDKVIPACLPSPNYVVADRTECFITGWGETQGTFGAGLLKEAQLPVIENKVCNRYEFLNGRVQSTELCAGHLAGGTDSCQGDSGGPLVCFEKDKYILQGVTSWGLGCARPNKPGVYVRVSRFVTWIEGVMRNN

SEQ ID NO: 9 - DNA, 1104 bp, 人工序列
  人工序列的描述：合成的多核苷酸
  Mini-plg(小纤维蛋白溶酶原)核酸序列
gtcaggtgggagtactgcaacctgaaaaaatgctcaggaacagaagcgagtgttgtagcacctccgcctgttgtcctgcttccagatgtagagactccttccgaagaagactgtatgtttgggaatgggaaaggataccgaggcaagagggcgaccactgttactgggacgccatgccaggactgggctgcccaggagccccatagacacagcattttcactccagagacaaatccacgggcgggtctggaaaaaaattactgccgtaaccctgatggtgatgtaggtggtccctggtgctacacgacaaatccaagaaaactttacgactactgtgatgtccctcagtgtgcggccccttcatttgattgtgggaagcctcaagtggagccgaagaaatgtcctggaagggttgtaggggggtgtgtggcccacccacattcctggccctggcaagtcagtcttagaacaaggtttggaatgcacttctgtggaggcaccttgatatccccagagtgggtgttgactgctgcccactgcttggagaagtccccaaggccttcatcctacaaggtcatcctgggtgcacaccaagaagtgaatctcgaaccgcatgttcaggaaatagaagtgtctaggctgttcttggagcccacacgaaaagatattgccttgctaaagctaagcagtcctgccgtcatcactgacaaagtaatcccagcttgtctgccatccccaaattatgtggtcgctgaccggaccgaatgtttcatcactggctggggagaaacccaaggtacttttggagctggccttctcaaggaagcccagctccctgtgattgagaataaagtgtgcaatcgctatgagtttctgaatggaagagtccaatccaccgaactctgtgctgggcatttggccggaggcactgacagttgccagggtgacagtggaggtcctctggtttgcttcgagaaggacaaatacattttacaaggagtcacttcttggggtcttggctgtgcacgccccaataagcctggtgtctatgttcgtgtttcaaggtttgttacttggattgagggagtgatgagaaataattaa

SEQ ID NO: 10 - protein, 367 aa, 人工序列
  人工序列的描述：合成的多肽
  Mini-plg(小纤维蛋白溶酶原)氨基酸序列
VRWEYCNLKKCSGTEASVVAPPPVVLLPDVETPSEEDCMFGNGKGYRGKRATTVTGTPCQDWAAQEPHRHSIFTPETNPRAGLEKNYCRNPDGDVGGPWCYTTNPRKLYDYCDVPQCAAPSFDCGKPQVEPKKCPGRVVGGCVAHPHSWPWQVSLRTRFGMHFCGGTLISPEWVLTAAHCLEKSPRPSSYKVILGAHQEVNLEPHVQEIEVSRLFLEPTRKDIALLKLSSPAVITDKVIPACLPSPNYVVADRTECFITGWGETQGTFGAGLLKEAQLPVIENKVCNRYEFLNGRVQSTELCAGHLAGGTDSCQGDSGGPLVCFEKDKYILQGVTSWGLGCARPNKPGVYVRVSRFVTWIEGVMRNN

SEQ ID NO: 11 - DNA, 750 bp, 人工序列
  人工序列的描述：合成的多核苷酸
  Micro-plg(微纤维蛋白溶酶原)核酸序列
gccccttcatttgattgtgggaagcctcaagtggagccgaagaaatgtcctggaagggttgtaggggggtgtgtggcccacccacattcctggccctggcaagtcagtcttagaacaaggtttggaatgcacttctgtggaggcaccttgatatccccagagtgggtgttgactgctgcccactgcttggagaagtccccaaggccttcatcctacaaggtcatcctgggtgcacaccaagaagtgaatctcgaaccgcatgttcaggaaatagaagtgtctaggctgttcttggagcccacacgaaaagatattgccttgctaaagctaagcagtcctgccgtcatcactgacaaagtaatcccagcttgtctgccatccccaaattatgtggtcgctgaccggaccgaatgtttcatcactggctggggagaaacccaaggtacttttggagctggccttctcaaggaagcccagctccctgtgattgagaataaagtgtgcaatcgctatgagtttctgaatggaagagtccaatccaccgaactctgtgctgggcatttggccggaggcactgacagttgccagggtgacagtggaggtcctctggtttgcttcgagaaggacaaatacattttacaaggagtcacttcttggggtcttggctgtgcacgccccaataagcctggtgtctatgttcgtgtttcaaggtttgttacttggattgagggagtgatgagaaataattaa

SEQ ID NO: 12 - protein, 249 aa, 人工序列
  人工序列的描述：合成的多肽
  Micro-plg(微纤维蛋白溶酶原)氨基酸序列
APSFDCGKPQVEPKKCPGRVVGGCVAHPHSWPWQVSLRTRFGMHFCGGTLISPEWVLTAAHCLEKSPRPSSYKVILGAHQEVNLEPHVQEIEVSRLFLEPTRKDIALLKLSSPAVITDKVIPACLPSPNYVVADRTECFITGWGETQGTFGAGLLKEAQLPVIENKVCNRYEFLNGRVQSTELCAGHLAGGTDSCQGDSGGPLVCFEKDKYILQGVTSWGLGCARPNKPGVYVRVSRFVTWIEGVMRNN

SEQ ID NO: 13 - DNA, 684 bp, 人工序列
  人工序列的描述：合成的多核苷酸
  丝氨酸蛋白酶(结构)域的核酸序列
gttgtaggggggtgtgtggcccacccacattcctggccctggcaagtcagtcttagaacaaggtttggaatgcacttctgtggaggcaccttgatatccccagagtgggtgttgactgctgcccactgcttggagaagtccccaaggccttcatcctacaaggtcatcctgggtgcacaccaagaagtgaatctcgaaccgcatgttcaggaaatagaagtgtctaggctgttcttggagcccacacgaaaagatattgccttgctaaagctaagcagtcctgccgtcatcactgacaaagtaatcccagcttgtctgccatccccaaattatgtggtcgctgaccggaccgaatgtttcatcactggctggggagaaacccaaggtacttttggagctggccttctcaaggaagcccagctccctgtgattgagaataaagtgtgcaatcgctatgagtttctgaatggaagagtccaatccaccgaactctgtgctgggcatttggccggaggcactgacagttgccagggtgacagtggaggtcctctggtttgcttcgagaaggacaaatacattttacaaggagtcacttcttggggtcttggctgtgcacgccccaataagcctggtgtctatgttcgtgtttcaaggtttgttacttggattgagggagtgatgaga

SEQ ID NO: 14 - protein, 228 aa, 人工序列
  人工序列的描述：合成的多肽
  丝氨酸蛋白酶(结构)域的氨基酸序列
VVGGCVAHPHSWPWQVSLRTRFGMHFCGGTLISPEWVLTAAHCLEKSPRPSSYKVILGAHQEVNLEPHVQEIEVSRLFLEPTRKDIALLKLSSPAVITDKVIPACLPSPNYVVADRTECFITGWGETQGTFGAGLLKEAQLPVIENKVCNRYEFLNGRVQSTELCAGHLAGGTDSCQGDSGGPLVCFEKDKYILQGVTSWGLGCARPNKPGVYVRVSRFVTWIEGVMR

SEQ ID NO: 15 - DNA, 20 bp, 人工序列
  人工序列的描述：合成的多核苷酸
  正向引物
gcggcggcagtggtggcggc

SEQ ID NO: 16 - DNA, 22 bp, 人工序列
  人工序列的描述：合成的多核苷酸
  反向引物
agtagatcggacagattttgct